European Patent Specification EP 3 404 101 B1, published June 11, 2025. Title: Method of producing L-lysine using microorganism having ability to produce L-lysine. Applicant: CJ CheilJedang Corporation. The sequence listing filed with the application follows.

SEQUENCE LISTING (18 sequences)

SEQ ID NO: 1 - DNA, 36 bp, Artificial Sequence
  primer lysC/ATG/FX
ccggggatcctctagacttagggagccatcttttgg

SEQ ID NO: 2 - DNA, 18 bp, Artificial Sequence
  primer lysC/ATG/R
ccagggccatctttgtgc

SEQ ID NO: 3 - DNA, 18 bp, Artificial Sequence
  primer lysC/ATG/F
gcacaaagatggccctgg

SEQ ID NO: 4 - DNA, 36 bp, Artificial Sequence
  primer lysC/ATG/RX
gcaggtcgactctagaagtgacatcaacaatgcgtg

SEQ ID NO: 5 - DNA, 36 bp, Artificial Sequence
  primer tkt/ATG/FX
ccggggatcctctagagaaatagatgggtgtagacg

SEQ ID NO: 6 - DNA, 23 bp, Artificial Sequence
  primer tkt/ATG/R4
gtgacagcgtcatggtggtcaat

SEQ ID NO: 7 - DNA, 23 bp, Artificial Sequence
  primer tkt/ATG/F4
attgaccaccatgacgctgtcac

SEQ ID NO: 8 - DNA, 36 bp, Artificial Sequence
  primer tkt/ATG/RX
gcaggtcgactctagacgcagagccttcaggtcatc

SEQ ID NO: 9 - DNA, 36 bp, Artificial Sequence
  primer pyc/ATG/FX
ccggggatcctctagattttggggaaaagtgcaaag

SEQ ID NO: 10 - DNA, 19 bp, Artificial Sequence
  primer pyc/ATG/R
gagtcgacattagagtaat

SEQ ID NO: 11 - DNA, 19 bp, Artificial Sequence
  primer pyc/ATG/F
attactctaatgtcgactc

SEQ ID NO: 12 - DNA, 36 bp, Artificial Sequence
  primer pyc/ATG/RX
gcaggtcgactctagagggcattttcagacaggaag

SEQ ID NO: 13 - DNA, 1266 bp, Corynebacterium glutamicum lysC
gtggccctggtcgtacagaaatatggcggttcctcgcttgagagtgcggaacgcattagaaacgtcgctgaacggatcgttgccaccaagaaggctggaaatgatgtcgtggttgtctgctccgcaatgggagacaccacggatgaacttctagaacttgcagcggcagtgaatcccgttccgccagctcgtgaaatggatatgctcctgactgctggtgagcgtatttctaacgctctcgtcgccatggctattgagtcccttggcgcagaagcccaatctttcacgggctctcaggctggtgtgctcaccaccgagcgccacggaaacgcacgcattgttgatgtcactccaggtcgtgtgcgtgaagcactcgatgagggcaagatctgcattgttgctggtttccagggtgttaataaagaaacccgcgatgtcaccacgttgggtcgtggtggttctgacaccactgcagttgcgttggcagctgctttgaacgctgatgtgtgtgagatttactcggacgttgacggtgtgtataccgctgacccgcgcatcgttcctaatgcacagaagctggaaaagctcagcttcgaagaaatgctggaacttgctgctgttggctccaagattttggtgctgcgcagtgttgaatacgctcgtgcattcaatgtgccacttcgcgtacgctcgtcttatagtaatgatcccggcactttgattgccggctctatggaggatattcctgtggaagaagcagtccttaccggtgtcgcaaccgacaagtccgaagccaaagtaaccgttctgggtatttccgataagccaggcgaggctgcgaaggttttccgtgcgttggctgatgcagaaatcaacattgacatggttctgcagaacgtctcttctgtagaagacggcaccaccgacatcaccttcacctgccctcgttccgacggccgccgcgcgatggagatcttgaagaagcttcaggttcagggcaactggaccaatgtgctttacgacgaccaggtcggcaaagtctccctcgtgggtgctggcatgaagtctcacccaggtgttaccgcagagttcatggaagctctgcgcgatgtcaacgtgaacatcgaattgatttccacctctgagattcgtatttccgtgctgatccgtgaagatgatctggatgctgctgcacgtgcattgcatgagcagttccagctgggcggcgaagacgaagccgtcgtttatgcaggcaccggacgctaa

SEQ ID NO: 14 - DNA, 2094 bp, Corynebacterium glutamicum tkt
ttgacgctgtcacctgaacttcaggcgctcactgtacgcaattacccctctgattggtccgatgtggacaccaaggctgtagacactgttcgtgtcctcgctgcagacgctgtagaaaactgtggctccggccacccaggcaccgcaatgagcctggctccccttgcatacaccttgtaccagcgggttatgaacgtagatccacaggacaccaactgggcaggccgtgaccgcttcgttctttcttgtggccactcctctttgacccagtacatccagctttacttgggtggattcggccttgagatggatgacctgaaggctctgcgcacctgggattccttgaccccaggacaccctgagtaccgccacaccaagggcgttgagatcaccactggccctcttggccagggtcttgcatctgcagttggtatggccatggctgctcgtcgtgagcgtggcctattcgacccaaccgctgctgagggcgaatccccattcgaccaccacatctacgtcattgcttctgatggtgacctgcaggaaggtgtcacctctgaggcatcctccatcgctggcacccagcagctgggcaacctcatcgtgttctgggatgacaaccgcatctccatcgaagacaacactgagatcgctttcaacgaggacgttgttgctcgttacaaggcttacggctggcagaccattgaggttgaggctggcgaggacgttgcagcaatcgaagctgcagtggctgaggctaagaaggacaccaagcgacctaccttcatccgcgttcgcaccatcatcggcttcccagctccaactatgatgaacaccggtgctgtgcacggtgctgctcttggcgcagctgaggttgcagcaaccaagactgagcttggattcgatcctgaggctcacttcgcgatcgacgatgaggttatcgctcacacccgctccctcgcagagcgcgctgcacagaagaaggctgcatggcaggtcaagttcgatgagtgggcagctgccaaccctgagaacaaggctctgttcgatcgcctgaactcccgtgagcttccagcgggctacgctgacgagctcccaacatgggatgcagatgagaagggcgtcgcaactcgtaaggcttccgaggctgcacttcaggcactgggcaagacccttcctgagctgtggggcggttccgctgacctcgcaggttccaacaacaccgtgatcaagggctccccttccttcggccctgagtccatctccaccgagacctggtctgctgagccttacggccgtaacctgcacttcggtatccgtgagcacgctatgggatccatcctcaacggcatttccctccacggtggcacccgcccatacggcggaaccttcctcatcttctccgactacatgcgtcctgcagttcgtcttgcagctctcatggagaccgacgcttactacgtctggacccacgactccatcggtctgggcgaagatggcccaacccaccagcctgttgaaaccttggctgcactgcgcgccatcccaggtctgtccgtcctgcgtcctgcagatgcgaacgagaccgcccaggcttgggctgcagcacttgagtacaaggaaggccctaagggtcttgcactgacccgccagaacgttcctgttctggaaggcaccaaggagaaggctgctgaaggcgttcgccgcggtggctacgtcctggttgagggttccaaggaaaccccagatgtgatcctcatgggctccggctccgaggttcagcttgcagttaacgctgcgaaggctctggaagctgagggcgttgcagctcgcgttgtttccgttccttgcatggattggttccaggagcaggacgcagagtacatcgagtccgttctgcctgcagctgtgaccgctcgtgtgtctgttgaagctggcatcgcaatgccttggtaccgcttcttgggcacccagggccgtgctgtctcccttgagcacttcggtgcttctgcggattaccagaccctgtttgagaagttcggcatcaccaccgatgcagtcgtggcagcggccaaggactccattaacggttaa

SEQ ID NO: 15 - DNA, 3423 bp, Corynebacterium glutamicum pyc
gtgtcgactcacacatcttcaacgcttccagcattcaaaaagatcttggtagcaaaccgcggcgaaatcgcggtccgtgctttccgtgcagcactcgaaaccggtgcagccacggtagctatttacccccgtgaagatcggggatcattccaccgctcttttgcttctgaagctgtccgcattggtaccgaaggctcaccagtcaaggcgtacctggacatcgatgaaattatcggtgcagctaaaaaagttaaagcagatgccatttacccgggatacggcttcctgtctgaaaatgcccagcttgcccgcgagtgtgcggaaaacggcattacttttattggcccaaccccagaggttcttgatctcaccggtgataagtctcgcgcggtaaccgccgcgaagaaggctggtctgccagttttggcggaatccaccccgagcaaaaacatcgatgagatcgttaaaagcgctgaaggccagacttaccccatctttgtgaaggcagttgccggtggtggcggacgcggtatgcgttttgttgcttcacctgatgagcttcgcaaattagcaacagaagcatctcgtgaagctgaagcggctttcggcgatggcgcggtatatgtcgaacgtgctgtgattaaccctcagcatattgaagtgcagatccttggcgatcacactggagaagttgtacacctttatgaacgtgactgctcactgcagcgtcgtcaccaaaaagttgtcgaaattgcgccagcacagcatttggatccagaactgcgtgatcgcatttgtgcggatgcagtaaagttctgccgctccattggttaccagggcgcgggaaccgtggaattcttggtcgatgaaaagggcaaccacgtcttcatcgaaatgaacccacgtatccaggttgagcacaccgtgactgaagaagtcaccgaggtggacctggtgaaggcgcagatgcgcttggctgctggtgcaaccttgaaggaattgggtctgacccaagataagatcaagacccacggtgcagcactgcagtgccgcatcaccacggaagatccaaacaacggcttccgcccagataccggaactatcaccgcgtaccgctcaccaggcggagctggcgttcgtcttgacggtgcagctcagctcggtggcgaaatcaccgcacactttgactccatgctggtgaaaatgacctgccgtggttccgactttgaaactgctgttgctcgtgcacagcgcgcgttggctgagttcaccgtgtctggtgttgcaaccaacattggtttcttgcgtgcgttgctgcgggaagaggacttcacttccaagcgcatcgccaccggattcattgccgatcacccgcacctccttcaggctccacctgctgatgatgagcagggacgcatcctggattacttggcagatgtcaccgtgaacaagcctcatggtgtgcgtccaaaggatgttgcagctcctatcgataagctgcctaacatcaaggatctgccactgccacgcggttcccgtgaccgcctgaagcagcttggcccagccgcgtttgctcgtgatctccgtgagcaggacgcactggcagttactgataccaccttccgcgatgcacaccagtctttgcttgcgacccgagtccgctcattcgcactgaagcctgcggcagaggccgtcgcaaagctgactcctgagcttttgtccgtggaggcctggggcggcgcgacctacgatgtggcgatgcgtttcctctttgaggatccgtgggacaggctcgacgagctgcgcgaggcgatgccgaatgtaaacattcagatgctgcttcgcggccgcaacaccgtgggatacaccccgtacccagactccgtctgccgcgcgtttgttaaggaagctgccagctccggcgtggacatcttccgcatcttcgacgcgcttaacgacgtctcccagatgcgtccagcaatcgacgcagtcctggagaccaacaccgcggtagccgaggtggctatggcttattctggtgatctctctgatccaaatgaaaagctctacaccctggattactacctaaagatggcagaggagatcgtcaagtctggcgctcacatcttggccattaaggatatggctggtctgcttcgcccagctgcggtaaccaagctggtcaccgcactgcgccgtgaattcgatctgccagtgcacgtgcacacccacgacactgcgggtggccagctggcaacctactttgctgcagctcaagctggtgcagatgctgttgacggtgcttccgcaccactgtctggcaccacctcccagccatccctgtctgccattgttgctgcattcgcgcacacccgtcgcgataccggtttgagcctcgaggctgtttctgacctcgagccgtactgggaagcagtgcgcggactgtacctgccatttgagtctggaaccccaggcccaaccggtcgcgtctaccgccacgaaatcccaggcggacagttgtccaacctgcgtgcacaggccaccgcactgggccttgcggatcgtttcgaactcatcgaagacaactacgcagccgttaatgagatgctgggacgcccaaccaaggtcaccccatcctccaaggttgttggcgacctcgcactccacctcgttggtgcgggtgtggatccagcagactttgctgccgatccacaaaagtacgacatcccagactctgtcatcgcgttcctgcgcggcgagcttggtaaccctccaggtggctggccagagccactgcgcacccgcgcactggaaggccgctccgaaggcaaggcacctctgacggaagttcctgaggaagagcaggcgcacctcgacgctgatgattccaaggaacgtcgcaatagcctcaaccgcctgctgttcccgaagccaaccgaagagttcctcgagcaccgtcgccgcttcggcaacacctctgcgctggatgatcgtgaattcttctacggcctggtcgaaggccgcgagactttgatccgcctgccagatgtgcgcaccccactgcttgttcgcctggatgcgatctctgagccagacgataagggtatgcgcaatgttgtggccaacgtcaacggccagatccgcccaatgcgtgtgcgtgaccgctccgttgagtctgtcaccgcaaccgcagaaaaggcagattcctccaacaagggccatgttgctgcaccattcgctggtgttgtcaccgtgactgttgctgaaggtgatgaggtcaaggctggagatgcagtcgcaatcatcgaggctatgaagatggaagcaacaatcactgcttctgttgacggcaaaatcgatcgcgttgtggttcctgctgcaacgaaggtggaaggtggcgacttgatcgtcgtcgtttcctaa

SEQ ID NO: 16 - DNA, 1266 bp, Artificial Sequence
  lysC with substituted start codon
atggccctggtcgtacagaaatatggcggttcctcgcttgagagtgcggaacgcattagaaacgtcgctgaacggatcgttgccaccaagaaggctggaaatgatgtcgtggttgtctgctccgcaatgggagacaccacggatgaacttctagaacttgcagcggcagtgaatcccgttccgccagctcgtgaaatggatatgctcctgactgctggtgagcgtatttctaacgctctcgtcgccatggctattgagtcccttggcgcagaagcccaatctttcacgggctctcaggctggtgtgctcaccaccgagcgccacggaaacgcacgcattgttgatgtcactccaggtcgtgtgcgtgaagcactcgatgagggcaagatctgcattgttgctggtttccagggtgttaataaagaaacccgcgatgtcaccacgttgggtcgtggtggttctgacaccactgcagttgcgttggcagctgctttgaacgctgatgtgtgtgagatttactcggacgttgacggtgtgtataccgctgacccgcgcatcgttcctaatgcacagaagctggaaaagctcagcttcgaagaaatgctggaacttgctgctgttggctccaagattttggtgctgcgcagtgttgaatacgctcgtgcattcaatgtgccacttcgcgtacgctcgtcttatagtaatgatcccggcactttgattgccggctctatggaggatattcctgtggaagaagcagtccttaccggtgtcgcaaccgacaagtccgaagccaaagtaaccgttctgggtatttccgataagccaggcgaggctgcgaaggttttccgtgcgttggctgatgcagaaatcaacattgacatggttctgcagaacgtctcttctgtagaagacggcaccaccgacatcaccttcacctgccctcgttccgacggccgccgcgcgatggagatcttgaagaagcttcaggttcagggcaactggaccaatgtgctttacgacgaccaggtcggcaaagtctccctcgtgggtgctggcatgaagtctcacccaggtgttaccgcagagttcatggaagctctgcgcgatgtcaacgtgaacatcgaattgatttccacctctgagattcgtatttccgtgctgatccgtgaagatgatctggatgctgctgcacgtgcattgcatgagcagttccagctgggcggcgaagacgaagccgtcgtttatgcaggcaccggacgctaa

SEQ ID NO: 17 - DNA, 2094 bp, Artificial Sequence
  tkt with substituted start codon
atgacgctgtcacctgaacttcaggcgctcactgtacgcaattacccctctgattggtccgatgtggacaccaaggctgtagacactgttcgtgtcctcgctgcagacgctgtagaaaactgtggctccggccacccaggcaccgcaatgagcctggctccccttgcatacaccttgtaccagcgggttatgaacgtagatccacaggacaccaactgggcaggccgtgaccgcttcgttctttcttgtggccactcctctttgacccagtacatccagctttacttgggtggattcggccttgagatggatgacctgaaggctctgcgcacctgggattccttgaccccaggacaccctgagtaccgccacaccaagggcgttgagatcaccactggccctcttggccagggtcttgcatctgcagttggtatggccatggctgctcgtcgtgagcgtggcctattcgacccaaccgctgctgagggcgaatccccattcgaccaccacatctacgtcattgcttctgatggtgacctgcaggaaggtgtcacctctgaggcatcctccatcgctggcacccagcagctgggcaacctcatcgtgttctgggatgacaaccgcatctccatcgaagacaacactgagatcgctttcaacgaggacgttgttgctcgttacaaggcttacggctggcagaccattgaggttgaggctggcgaggacgttgcagcaatcgaagctgcagtggctgaggctaagaaggacaccaagcgacctaccttcatccgcgttcgcaccatcatcggcttcccagctccaactatgatgaacaccggtgctgtgcacggtgctgctcttggcgcagctgaggttgcagcaaccaagactgagcttggattcgatcctgaggctcacttcgcgatcgacgatgaggttatcgctcacacccgctccctcgcagagcgcgctgcacagaagaaggctgcatggcaggtcaagttcgatgagtgggcagctgccaaccctgagaacaaggctctgttcgatcgcctgaactcccgtgagcttccagcgggctacgctgacgagctcccaacatgggatgcagatgagaagggcgtcgcaactcgtaaggcttccgaggctgcacttcaggcactgggcaagacccttcctgagctgtggggcggttccgctgacctcgcaggttccaacaacaccgtgatcaagggctccccttccttcggccctgagtccatctccaccgagacctggtctgctgagccttacggccgtaacctgcacttcggtatccgtgagcacgctatgggatccatcctcaacggcatttccctccacggtggcacccgcccatacggcggaaccttcctcatcttctccgactacatgcgtcctgcagttcgtcttgcagctctcatggagaccgacgcttactacgtctggacccacgactccatcggtctgggcgaagatggcccaacccaccagcctgttgaaaccttggctgcactgcgcgccatcccaggtctgtccgtcctgcgtcctgcagatgcgaacgagaccgcccaggcttgggctgcagcacttgagtacaaggaaggccctaagggtcttgcactgacccgccagaacgttcctgttctggaaggcaccaaggagaaggctgctgaaggcgttcgccgcggtggctacgtcctggttgagggttccaaggaaaccccagatgtgatcctcatgggctccggctccgaggttcagcttgcagttaacgctgcgaaggctctggaagctgagggcgttgcagctcgcgttgtttccgttccttgcatggattggttccaggagcaggacgcagagtacatcgagtccgttctgcctgcagctgtgaccgctcgtgtgtctgttgaagctggcatcgcaatgccttggtaccgcttcttgggcacccagggccgtgctgtctcccttgagcacttcggtgcttctgcggattaccagaccctgtttgagaagttcggcatcaccaccgatgcagtcgtggcagcggccaaggactccattaacggttaa

SEQ ID NO: 18 - DNA, 3423 bp, Artificial Sequence
  pyc with substituted start codon
atgtcgactcacacatcttcaacgcttccagcattcaaaaagatcttggtagcaaaccgcggcgaaatcgcggtccgtgctttccgtgcagcactcgaaaccggtgcagccacggtagctatttacccccgtgaagatcggggatcattccaccgctcttttgcttctgaagctgtccgcattggtaccgaaggctcaccagtcaaggcgtacctggacatcgatgaaattatcggtgcagctaaaaaagttaaagcagatgccatttacccgggatacggcttcctgtctgaaaatgcccagcttgcccgcgagtgtgcggaaaacggcattacttttattggcccaaccccagaggttcttgatctcaccggtgataagtctcgcgcggtaaccgccgcgaagaaggctggtctgccagttttggcggaatccaccccgagcaaaaacatcgatgagatcgttaaaagcgctgaaggccagacttaccccatctttgtgaaggcagttgccggtggtggcggacgcggtatgcgttttgttgcttcacctgatgagcttcgcaaattagcaacagaagcatctcgtgaagctgaagcggctttcggcgatggcgcggtatatgtcgaacgtgctgtgattaaccctcagcatattgaagtgcagatccttggcgatcacactggagaagttgtacacctttatgaacgtgactgctcactgcagcgtcgtcaccaaaaagttgtcgaaattgcgccagcacagcatttggatccagaactgcgtgatcgcatttgtgcggatgcagtaaagttctgccgctccattggttaccagggcgcgggaaccgtggaattcttggtcgatgaaaagggcaaccacgtcttcatcgaaatgaacccacgtatccaggttgagcacaccgtgactgaagaagtcaccgaggtggacctggtgaaggcgcagatgcgcttggctgctggtgcaaccttgaaggaattgggtctgacccaagataagatcaagacccacggtgcagcactgcagtgccgcatcaccacggaagatccaaacaacggcttccgcccagataccggaactatcaccgcgtaccgctcaccaggcggagctggcgttcgtcttgacggtgcagctcagctcggtggcgaaatcaccgcacactttgactccatgctggtgaaaatgacctgccgtggttccgactttgaaactgctgttgctcgtgcacagcgcgcgttggctgagttcaccgtgtctggtgttgcaaccaacattggtttcttgcgtgcgttgctgcgggaagaggacttcacttccaagcgcatcgccaccggattcattgccgatcacccgcacctccttcaggctccacctgctgatgatgagcagggacgcatcctggattacttggcagatgtcaccgtgaacaagcctcatggtgtgcgtccaaaggatgttgcagctcctatcgataagctgcctaacatcaaggatctgccactgccacgcggttcccgtgaccgcctgaagcagcttggcccagccgcgtttgctcgtgatctccgtgagcaggacgcactggcagttactgataccaccttccgcgatgcacaccagtctttgcttgcgacccgagtccgctcattcgcactgaagcctgcggcagaggccgtcgcaaagctgactcctgagcttttgtccgtggaggcctggggcggcgcgacctacgatgtggcgatgcgtttcctctttgaggatccgtgggacaggctcgacgagctgcgcgaggcgatgccgaatgtaaacattcagatgctgcttcgcggccgcaacaccgtgggatacaccccgtacccagactccgtctgccgcgcgtttgttaaggaagctgccagctccggcgtggacatcttccgcatcttcgacgcgcttaacgacgtctcccagatgcgtccagcaatcgacgcagtcctggagaccaacaccgcggtagccgaggtggctatggcttattctggtgatctctctgatccaaatgaaaagctctacaccctggattactacctaaagatggcagaggagatcgtcaagtctggcgctcacatcttggccattaaggatatggctggtctgcttcgcccagctgcggtaaccaagctggtcaccgcactgcgccgtgaattcgatctgccagtgcacgtgcacacccacgacactgcgggtggccagctggcaacctactttgctgcagctcaagctggtgcagatgctgttgacggtgcttccgcaccactgtctggcaccacctcccagccatccctgtctgccattgttgctgcattcgcgcacacccgtcgcgataccggtttgagcctcgaggctgtttctgacctcgagccgtactgggaagcagtgcgcggactgtacctgccatttgagtctggaaccccaggcccaaccggtcgcgtctaccgccacgaaatcccaggcggacagttgtccaacctgcgtgcacaggccaccgcactgggccttgcggatcgtttcgaactcatcgaagacaactacgcagccgttaatgagatgctgggacgcccaaccaaggtcaccccatcctccaaggttgttggcgacctcgcactccacctcgttggtgcgggtgtggatccagcagactttgctgccgatccacaaaagtacgacatcccagactctgtcatcgcgttcctgcgcggcgagcttggtaaccctccaggtggctggccagagccactgcgcacccgcgcactggaaggccgctccgaaggcaaggcacctctgacggaagttcctgaggaagagcaggcgcacctcgacgctgatgattccaaggaacgtcgcaatagcctcaaccgcctgctgttcccgaagccaaccgaagagttcctcgagcaccgtcgccgcttcggcaacacctctgcgctggatgatcgtgaattcttctacggcctggtcgaaggccgcgagactttgatccgcctgccagatgtgcgcaccccactgcttgttcgcctggatgcgatctctgagccagacgataagggtatgcgcaatgttgtggccaacgtcaacggccagatccgcccaatgcgtgtgcgtgaccgctccgttgagtctgtcaccgcaaccgcagaaaaggcagattcctccaacaagggccatgttgctgcaccattcgctggtgttgtcaccgtgactgttgctgaaggtgatgaggtcaaggctggagatgcagtcgcaatcatcgaggctatgaagatggaagcaacaatcactgcttctgttgacggcaaaatcgatcgcgttgtggttcctgctgcaacgaaggtggaaggtggcgacttgatcgtcgtcgtttcctaa